European Patent Application EP 4 183 421 A1, published May 24, 2023. Title: ANTIBODY DRUG CONJUGATE. Applicant: CHIA TAI TIANQING PHARMACEUTICAL GROUP CO., LTD. NANJING SHUNXIN PHARMACEUTICALS CO., LTD. OF CHIATAI TIANQING PHARMACEUTICAL GROUP. The sequence listing filed with the application follows.

SEQUENCE LISTING (50 sequences)

SEQ ID NO: 1 - protein, 475 aa, Artificial Sequence
  Amino acid sequence of anti-Her2 scFv-Fc
EVQLVESGGGLVQPGGSLRLSCAASGFNIKDTYIHWVRQAPGKGLEWVARIYPTNGYTRYADSVKGRFTISADTSKNTAYLQMNSLRAEDTAVYYCSRWGGDGFYAMDYWGQGTLVTVSSGGGGSGGGGSGGGGSDIQMTQSPSSLSASVGDRVTITCRASQDVNTAVAWYQQKPGKAPKLLIYSASFLYSGVPSRFSGSRSGTDFTLTISSLQPEDFATYYCQQHYTTPPTFGQGTKVEIKGEPKSSDKTHTCPPCPAPELLGGPSVFLFPPKPKDTLMISRTPEVTCVVVDVSHEDPEVKFNWYVDGVEVHNAKTKPREEQYNSTYRVVSVLTVLHQDWLNGKEYKCKVSNKALPAPIEKTISKAKGQPREPQVYTLPPSREEMTKNQVSLTCLVKGFYPSDIAVEWESNGQPENNYKTTPPVLDSDGSFFLYSKLTVDKSRWQQGNVFSCSVMHEALHNHYTQKSLSLSPGK

SEQ ID NO: 2 - DNA, 1425 bp, Artificial Sequence
  Encoding DNA sequence of anti-Her2 scFv-Fc
gaggtgcagctggtggagtctggaggaggactggtgcagccaggaggcagcctgcggctgtcttgtgccgcttccggcttcaacatcaaggacacctacatccattgggtgaggcaggctccaggcaagggactggagtgggtggctcggatctatcctaccaatggctacacaagatatgccgactccgtgaagggccggtttaccatcagcgccgatacctctaagaacacagcttacctgcagatgaattccctgagggccgaggacacagccgtgtactattgcagcagatggggaggcgacggcttctacgctatggattattggggccagggcaccctggtgacagtgtccagcggcggcggcggctctggaggaggaggatccggaggaggaggaagcgatatccagatgacccagtccccttcttccctgtctgcctccgtgggcgacagagtgaccatcacatgtcgcgctagccaggatgtgaacacagccgtggcttggtaccagcagaagccaggcaaggcccccaagctgctgatctactccgcctccttcctgtattccggagtgccaagcaggttttccggaagccggtctggaaccgacttcaccctgacaatcagctctctgcagcctgaggattttgccacatactattgccagcagcactataccacaccccctaccttcggccagggcacaaaggtggagatcaagggcgagccaaagtccagcgacaagacccatacatgcccaccatgtcctgctccagagctgctgggcggcccttccgtgttcctgtttcctccaaagccaaaggataccctgatgatctctagaacccctgaggtgacatgcgtggtggtggacgtgtcccacgaggatccagaggtgaagtttaactggtacgtggacggcgtggaggtgcataatgccaagaccaagccaagagaggagcagtacaattctacctatcgcgtggtgtccgtgctgacagtgctgcaccaggattggctgaacggcaaggagtataagtgcaaggtgagcaataaggccctgcccgctcccatcgagaagaccatctctaaggctaagggccagcccagagagcctcaggtgtacacactgccccctagccgcgaggagatgaccaagaaccaggtgtctctgacatgtctggtgaagggcttttatccatctgacatcgccgtggagtgggagtccaatggccagcccgagaacaattacaagaccacaccacccgtgctggactctgatggctccttctttctgtattccaagctgaccgtggataagagccgctggcagcagggcaacgtgttctcctgcagcgtgatgcatgaggctctgcacaatcattacacacagaagtctctgtccctgagccctggcaag

SEQ ID NO: 3 - protein, 475 aa, Artificial Sequence
  Amino acid sequence of anti-Her2-scFv-VL-F53Y-Fc
EVQLVESGGGLVQPGGSLRLSCAASGFNIKDTYIHWVRQAPGKGLEWVARIYPTNGYTRYADSVKGRFTISADTSKNTAYLQMNSLRAEDTAVYYCSRWGGDGFYAMDYWGQGTLVTVSSGGGGSGGGGSGGGGSDIQMTQSPSSLSASVGDRVTITCRASQDVNTAVAWYQQKPGKAPKLLIYSASYLYSGVPSRFSGSRSGTDFTLTISSLQPEDFATYYCQQHYTTPPTFGQGTKVEIKGEPKSSDKTHTCPPCPAPELLGGPSVFLFPPKPKDTLMISRTPEVTCVVVDVSHEDPEVKFNWYVDGVEVHNAKTKPREEQYNSTYRVVSVLTVLHQDWLNGKEYKCKVSNKALPAPIEKTISKAKGQPREPQVYTLPPSREEMTKNQVSLTCLVKGFYPSDIAVEWESNGQPENNYKTTPPVLDSDGSFFLYSKLTVDKSRWQQGNVFSCSVMHEALHNHYTQKSLSLSPGK

SEQ ID NO: 4 - DNA, 1425 bp, Artificial Sequence
  Encoding DNA sequence of anti-Her2-scFv-VL-F53Y-Fc
gaggtgcagctggtggagtctggaggaggactggtgcagccaggaggcagcctgcggctgtcttgtgccgcttccggcttcaacatcaaggacacctacatccattgggtgaggcaggctccaggcaagggactggagtgggtggctcggatctatcctaccaatggctacacaagatatgccgactccgtgaagggccggtttaccatcagcgccgatacctctaagaacacagcttacctgcagatgaattccctgagggccgaggacacagccgtgtactattgcagcagatggggaggcgacggcttctacgctatggattattggggccagggcaccctggtgacagtgtccagcggcggcggcggctctggaggaggaggatccggaggaggaggaagcgatatccagatgacccagtccccttcttccctgtctgcctccgtgggcgacagagtgaccatcacatgtcgcgctagccaggatgtgaacacagccgtggcttggtaccagcagaagccaggcaaggcccccaagctgctgatctactccgcctcctacctgtattccggagtgccaagcaggttttccggaagccggtctggaaccgacttcaccctgacaatcagctctctgcagcctgaggattttgccacatactattgccagcagcactataccacaccccctaccttcggccagggcacaaaggtggagatcaagggcgagccaaagtccagcgacaagacccatacatgcccaccatgtcctgctccagagctgctgggcggcccttccgtgttcctgtttcctccaaagccaaaggataccctgatgatctctagaacccctgaggtgacatgcgtggtggtggacgtgtcccacgaggatccagaggtgaagtttaactggtacgtggacggcgtggaggtgcataatgccaagaccaagccaagagaggagcagtacaattctacctatcgcgtggtgtccgtgctgacagtgctgcaccaggattggctgaacggcaaggagtataagtgcaaggtgagcaataaggccctgcccgctcccatcgagaagaccatctctaaggctaagggccagcccagagagcctcaggtgtacacactgccccctagccgcgaggagatgaccaagaaccaggtgtctctgacatgtctggtgaagggcttttatccatctgacatcgccgtggagtgggagtccaatggccagcccgagaacaattacaagaccacaccacccgtgctggactctgatggctccttctttctgtattccaagctgaccgtggataagagccgctggcagcagggcaacgtgttctcctgcagcgtgatgcatgaggctctgcacaatcattacacacagaagtctctgtccctgagccctggcaag

SEQ ID NO: 5 - protein, 475 aa, Artificial Sequence
  Amino acid sequence of anti-Her2-scFv-VL-F53A-Fc
EVQLVESGGGLVQPGGSLRLSCAASGFNIKDTYIHWVRQAPGKGLEWVARIYPTNGYTRYADSVKGRFTISADTSKNTAYLQMNSLRAEDTAVYYCSRWGGDGFYAMDYWGQGTLVTVSSGGGGSGGGGSGGGGSDIQMTQSPSSLSASVGDRVTITCRASQDVNTAVAWYQQKPGKAPKLLIYSASALYSGVPSRFSGSRSGTDFTLTISSLQPEDFATYYCQQHYTTPPTFGQGTKVEIKGEPKSSDKTHTCPPCPAPELLGGPSVFLFPPKPKDTLMISRTPEVTCVVVDVSHEDPEVKFNWYVDGVEVHNAKTKPREEQYNSTYRVVSVLTVLHQDWLNGKEYKCKVSNKALPAPIEKTISKAKGQPREPQVYTLPPSREEMTKNQVSLTCLVKGFYPSDIAVEWESNGQPENNYKTTPPVLDSDGSFFLYSKLTVDKSRWQQGNVFSCSVMHEALHNHYTQKSLSLSPGK

SEQ ID NO: 6 - DNA, 1425 bp, Artificial Sequence
  Encoding DNA sequence of anti-Her2-scFv-VL-F53A-Fc
gaggtgcagctggtggagtctggaggaggactggtgcagccaggaggcagcctgcggctgtcttgtgccgcttccggcttcaacatcaaggacacctacatccattgggtgaggcaggctccaggcaagggactggagtgggtggctcggatctatcctaccaatggctacacaagatatgccgactccgtgaagggccggtttaccatcagcgccgatacctctaagaacacagcttacctgcagatgaattccctgagggccgaggacacagccgtgtactattgcagcagatggggaggcgacggcttctacgctatggattattggggccagggcaccctggtgacagtgtccagcggcggcggcggctctggaggaggaggatccggaggaggaggaagcgatatccagatgacccagtccccttcttccctgtctgcctccgtgggcgacagagtgaccatcacatgtcgcgctagccaggatgtgaacacagccgtggcttggtaccagcagaagccaggcaaggcccccaagctgctgatctactccgcctccgccctgtattccggagtgccaagcaggttttccggaagccggtctggaaccgacttcaccctgacaatcagctctctgcagcctgaggattttgccacatactattgccagcagcactataccacaccccctaccttcggccagggcacaaaggtggagatcaagggcgagccaaagtccagcgacaagacccatacatgcccaccatgtcctgctccagagctgctgggcggcccttccgtgttcctgtttcctccaaagccaaaggataccctgatgatctctagaacccctgaggtgacatgcgtggtggtggacgtgtcccacgaggatccagaggtgaagtttaactggtacgtggacggcgtggaggtgcataatgccaagaccaagccaagagaggagcagtacaattctacctatcgcgtggtgtccgtgctgacagtgctgcaccaggattggctgaacggcaaggagtataagtgcaaggtgagcaataaggccctgcccgctcccatcgagaagaccatctctaaggctaagggccagcccagagagcctcaggtgtacacactgccccctagccgcgaggagatgaccaagaaccaggtgtctctgacatgtctggtgaagggcttttatccatctgacatcgccgtggagtgggagtccaatggccagcccgagaacaattacaagaccacaccacccgtgctggactctgatggctccttctttctgtattccaagctgaccgtggataagagccgctggcagcagggcaacgtgttctcctgcagcgtgatgcatgaggctctgcacaatcattacacacagaagtctctgtccctgagccctggcaag

SEQ ID NO: 7 - protein, 475 aa, Artificial Sequence
  Amino acid sequence of anti-Her2-scFv-VL-F53R-Fc
EVQLVESGGGLVQPGGSLRLSCAASGFNIKDTYIHWVRQAPGKGLEWVARIYPTNGYTRYADSVKGRFTISADTSKNTAYLQMNSLRAEDTAVYYCSRWGGDGFYAMDYWGQGTLVTVSSGGGGSGGGGSGGGGSDIQMTQSPSSLSASVGDRVTITCRASQDVNTAVAWYQQKPGKAPKLLIYSASRLYSGVPSRFSGSRSGTDFTLTISSLQPEDFATYYCQQHYTTPPTFGQGTKVEIKGEPKSSDKTHTCPPCPAPELLGGPSVFLFPPKPKDTLMISRTPEVTCVVVDVSHEDPEVKFNWYVDGVEVHNAKTKPREEQYNSTYRVVSVLTVLHQDWLNGKEYKCKVSNKALPAPIEKTISKAKGQPREPQVYTLPPSREEMTKNQVSLTCLVKGFYPSDIAVEWESNGQPENNYKTTPPVLDSDGSFFLYSKLTVDKSRWQQGNVFSCSVMHEALHNHYTQKSLSLSPGK

SEQ ID NO: 8 - DNA, 1427 bp, Artificial Sequence
  Encoding DNA sequence of anti-Her2-scFv-VL-F53R-Fc
gaggtgcagctggtggagtctggaggaggactggtgcagccaggaggcagcctgcggctgtcttgtgccgcttccggcttcaacatcaaggacacctacatccattgggtgaggcaggctccaggcaagggactggagtgggtggctcggatctatcctaccaatggctacacaagatatgccgactccgtgaagggccggtttaccatcagcgccgatacctctaagaacacagcttacctgcagatgaattccctgagggccgaggacacagccgtgtactattgcagcagatggggaggcgacggcttctacgctatggattattggggccagggcaccctggtgacagtgtccagcggcggcggcggctctggaggaggaggatccggaggaggaggaagcgatatccagatgacccagtccccttcttccctgtctgcctccgtgggcgacagagtgaccatcacatgtcgcgctagccaggatgtgaacacagccgtggcttggtaccagcagaagccaggcaaggcccccaagctgctgatctactccgcctccaggctgtattccggagtgccaagcaggttttccggaagccggtctggaaccgacttcaccctgacaatcagctctctgcagcctgaggattttgccacatactattgccagcagcactataccacaccccctaccttcggccagggcacaaaggtggagatcaagggcgagccaaagtccagcgacaagacccatacatgcccaccatgtcctgctccagagctgctgggcggcccttccgtgttcctgtttcctccaaagccaaaggataccctgatgatctctagaacccctgaggtgacatgcgtggtggtggacgtgtcccacgaggatccagaggtgaagtttaactggtacgtggacggcgtggaggtgcataatgccaagaccaagccaagagaggagcagtacaattctacctatcgcgtggtgtccgtgctgacagtgctgcaccaggattggctgaacggcaaggagtataagtgcaaggtgagcaataaggccctgcccgctcccatcgagaagaccatctctaaggctaagggccagcccagagagcctcaggtgtacacactgccccctagccgcgaggagatgaccaagaaccaggtgtctctgacatgtctggtgaagggcttttatccatctgacatcgccgtggagtgggagtccaatggccagcccgagaacaattacaagaccacaccacccgtgctggactctgatggctccttctttctgtattccaagctgaccgtggataagagccgctggcagcagggcaacgtgttctcctgcagcgtgatgcatgaggctctgcacaatcattacacacagaagtctctgtccctgagccctggcaagta

SEQ ID NO: 9 - protein, 475 aa, Artificial Sequence
  Amino acid sequence of anti-Her2-scFv-VH-K30E-Fc
EVQLVESGGGLVQPGGSLRLSCAASGFNIEDTYIHWVRQAPGKGLEWVARIYPTNGYTRYADSVKGRFTISADTSKNTAYLQMNSLRAEDTAVYYCSRWGGDGFYAMDYWGQGTLVTVSSGGGGSGGGGSGGGGSDIQMTQSPSSLSASVGDRVTITCRASQDVNTAVAWYQQKPGKAPKLLIYSASFLYSGVPSRFSGSRSGTDFTLTISSLQPEDFATYYCQQHYTTPPTFGQGTKVEIKGEPKSSDKTHTCPPCPAPELLGGPSVFLFPPKPKDTLMISRTPEVTCVVVDVSHEDPEVKFNWYVDGVEVHNAKTKPREEQYNSTYRVVSVLTVLHQDWLNGKEYKCKVSNKALPAPIEKTISKAKGQPREPQVYTLPPSREEMTKNQVSLTCLVKGFYPSDIAVEWESNGQPENNYKTTPPVLDSDGSFFLYSKLTVDKSRWQQGNVFSCSVMHEALHNHYTQKSLSLSPGK

SEQ ID NO: 10 - DNA, 1425 bp, Artificial Sequence
  Encoding DNA sequence of anti-Her2-scFv-VH-K30E-Fc
gaggtgcagctggtggagtctggaggaggactggtgcagccaggaggcagcctgcggctgtcttgtgccgcttccggcttcaacatcgaggacacctacatccattgggtgaggcaggctccaggcaagggactggagtgggtggctcggatctatcctaccaatggctacacaagatatgccgactccgtgaagggccggtttaccatcagcgccgatacctctaagaacacagcttacctgcagatgaattccctgagggccgaggacacagccgtgtactattgcagcagatggggaggcgacggcttctacgctatggattattggggccagggcaccctggtgacagtgtccagcggcggcggcggctctggaggaggaggatccggaggaggaggaagcgatatccagatgacccagtccccttcttccctgtctgcctccgtgggcgacagagtgaccatcacatgtcgcgctagccaggatgtgaacacagccgtggcttggtaccagcagaagccaggcaaggcccccaagctgctgatctactccgcctccttcctgtattccggagtgccaagcaggttttccggaagccggtctggaaccgacttcaccctgacaatcagctctctgcagcctgaggattttgccacatactattgccagcagcactataccacaccccctaccttcggccagggcacaaaggtggagatcaagggcgagccaaagtccagcgacaagacccatacatgcccaccatgtcctgctccagagctgctgggcggcccttccgtgttcctgtttcctccaaagccaaaggataccctgatgatctctagaacccctgaggtgacatgcgtggtggtggacgtgtcccacgaggatccagaggtgaagtttaactggtacgtggacggcgtggaggtgcataatgccaagaccaagccaagagaggagcagtacaattctacctatcgcgtggtgtccgtgctgacagtgctgcaccaggattggctgaacggcaaggagtataagtgcaaggtgagcaataaggccctgcccgctcccatcgagaagaccatctctaaggctaagggccagcccagagagcctcaggtgtacacactgccccctagccgcgaggagatgaccaagaaccaggtgtctctgacatgtctggtgaagggcttttatccatctgacatcgccgtggagtgggagtccaatggccagcccgagaacaattacaagaccacaccacccgtgctggactctgatggctccttctttctgtattccaagctgaccgtggataagagccgctggcagcagggcaacgtgttctcctgcagcgtgatgcatgaggctctgcacaatcattacacacagaagtctctgtccctgagccctggcaag

SEQ ID NO: 11 - protein, 480 aa, Artificial Sequence
  Amino acid sequence of anti-Her2-scFv-VH-K30E-VL-F53Y-Fc
EVQLVESGGGLVQPGGSLRLSCAASGFNIEDTYIHWVRQAPGKGLEWVARIYPTNGYTRYADSVKGRFTISADTSKNTAYLQMNSLRAEDTAVYYCSRWGGDGFYAMDYWGQGTLVTVSSGGGGSGGGGSGGGGSGGGGSDIQMTQSPSSLSASVGDRVTITCRASQDVNTAVAWYQQKPGKAPKLLIYSASYLYSGVPSRFSGSRSGTDFTLTISSLQPEDFATYYCQQHYTTPPTFGQGTKVEIKGEPKSSDKTHTCPPCPAPELLGGPSVFLFPPKPKDTLMISRTPEVTCVVVDVSHEDPEVKFNWYVDGVEVHNAKTKPREEQYNSTYRVVSVLTVLHQDWLNGKEYKCKVSNKALPAPIEKTISKAKGQPREPQVYTLPPCREEMTKNQVSLWCLVKGFYPSDIAVEWESNGQPENNYKTTPPVLDSDGSFFLYSKLTVDKSRWQQGNVFSCSVMHEALHNHYTQKSLSLSPGK

SEQ ID NO: 12 - DNA, 1443 bp, Artificial Sequence
  Nucleotide sequence of anti-Her2-scFv-VH-K30E-VL-F53Y-Fc
gaggtgcaactggtggaatccggcgggggactggtccaacctggagggagcctgcggctgtcttgcgccgcctctggcttcaacatcgaggatacctacatccactgggtgcggcaggcccctggcaagggcctggaatgggtcgctagaatctaccctaccaacggctacaccagatacgccgactctgtaaagggcagattcaccatctctgccgatacatctaagaacaccgcctacctgcagatgaactccctgagagccgaggacaccgccgtgtactactgctcccggtggggcggtgacggcttttacgccatggactactggggacaaggcacacttgttacggtgtcctctggaggcggcggctccggcggcggcggctctggcggaggcggctctggcggcggcggatctgatatccagatgacccagtctcctagctccctctccgcctccgtgggcgacagagtgacaatcacctgcagagcttctcaggacgtgaacaccgctgtggcctggtaccagcagaagcctggcaaggcccctaagctgctgatctactctgcttcctacctgtactccggcgtgcccagccggttctccggctctcggtccggcaccgacttcactctgaccatctccagcctgcagcctgaagatttcgccacctactactgccagcagcactacaccacccctcccaccttcggccagggcaccaaagtggagatcaagggcgagcccaagtcctccgataaaacccacacctgtcctccttgccctgcccctgaactactgggcggcccttctgtgttcctgttccctcctaagcccaaggacaccctgatgatctctagaacccctgaagtgacctgcgtggtggtggatgtgtctcacgaggaccctgaggtcaagttcaactggtacgtggacggcgtggaagtgcataacgccaagaccaagcctagagaagagcagtacaactccacctacagagtggtctccgtgctgaccgtgctgcaccaggactggctgaacggcaaagagtacaagtgcaaggtgtccaacaaggctctgcctgctcctatcgagaagacaatctccaaggccaaaggccagcctcgggagcctcaggtgtacaccctgcctccttgtagagaggaaatgaccaagaaccaggtgtctctgtggtgcctggtgaagggcttctacccatccgacatcgccgtcgagtgggagtccaacggacagcccgagaacaactacaagactaccccacctgtgctggactccgatggctccttcttcctgtactccaagctgaccgtggacaagtccagatggcagcagggcaacgtgttctcctgctccgtgatgcacgaggccctgcacaaccactacacccagaaatccctgtctctgtcccctggcaagtga

SEQ ID NO: 13 - protein, 449 aa, Artificial Sequence
  Amino acid sequence of anti-Her2-domain2-HC-Fc
EVQLVESGGGLVQPGGSLRLSCAASGFTFTDYTMDWVRQAPGKGLEWVADVNPNSGGSIYNQRFKGRFTLSVDRSKNTLYLQMNSLRAEDTAVYYCARNLGPSFYFDYWGQGTLVTVSSASTKGPSVFPLAPSSKSTSGGTAALGCLVKDYFPEPVTVSWNSGALTSGVHTFPAVLQSSGLYSLSSVVTVPSSSLGTQTYICNVNHKPSNTKVDKKVEPKSCDKTHTCPPCPAPELLGGPSVFLFPPKPKDTLMISRTPEVTCVVVDVSHEDPEVKFNWYVDGVEVHNAKTKPREEQYNSTYRVVSVLTVLHQDWLNGKEYKCKVSNKALPAPIEKTISKAKGQPREPQVCTLPPSREEMTKNQVSLSCAVKGFYPSDIAVEWESNGQPENNYKTTPPVLDSDGSFFLVSKLTVDKSRWQQGNVFSCSVMHEALHNRFTQKSLSLSPGK

SEQ ID NO: 14 - DNA, 1350 bp, Artificial Sequence
  Nucleotide sequence ofanti-Her2-domain2-HC-Fc
gaagtgcagctggttgaatctggcggcggattggttcagcctggcggatctctgagactgtcttgtgccgcctctggcttcaccttcaccgactacaccatggactgggtccgacaggctcctggcaaaggactggaatgggtcgccgacgtgaaccctaattccggcggctccatctacaaccagcggttcaagggcagattcaccctgtccgtggaccggtctaagaacaccctgtacctgcagatgaactccctgagagccgaggacaccgccgtgtactactgcgccagaaacctgggaccttccttctacttcgactactggggccagggcaccctggtcacagtttcttccgcttccaccaagggacccagcgtgttccctctggctccttccagcaagtctacctctggcggaacagctgctctgggctgcctggtcaaggactactttcctgagcctgtgaccgtgtcctggaactctggcgctctgacatctggcgtgcacacctttccagctgtgctgcagtcctccggcctgtactctctgtcctctgtcgtgaccgtgccttccagctctctgggaacccagacctacatctgcaatgtgaaccacaagccttccaacaccaaggtggacaagaaggtggaacccaagtcctgcgacaagacccacacctgtcctccatgtcctgctccagaactgctcggcggaccttccgtgttcctgtttcctccaaagcctaaggataccctgatgatctctcggacccctgaagtgacctgcgtggtggtggatgtgtctcacgaggatcccgaagtgaagttcaattggtacgtggacggcgtggaagtgcacaacgccaagaccaagcctagagaggaacagtacaactccacctacagagtggtgtccgtgctgaccgtgctgcaccaggattggctgaacggcaaagagtacaagtgcaaggtgtccaacaaggccctgcctgctcctatcgaaaagaccatctccaaggccaagggccagcctcgggaacctcaagtctgtaccctgcctcctagccgggaagagatgaccaagaaccaggtgtccctgtcctgtgccgtgaagggcttctacccttccgatatcgccgtggaatgggagagcaatggccagcctgagaacaactacaagacaacccctcctgtgctggactccgacggctcattcttcctggtgtccaagctgacagtggacaagtccagatggcagcagggcaacgtgttctcctgctccgtgatgcacgaggccctgcacaacaggttcacccagaagtccctgtctctgagccccggcaaatga

SEQ ID NO: 15 - protein, 214 aa, Artificial Sequence
  Amino acid sequence of anti-Her2-domain2-LC
DIQMTQSPSSLSASVGDRVTITCKASQDVSIGVAWYQQKPGKAPKLLIYSASYRYTGVPSRFSGSGSGTDFTLTISSLQPEDFATYYCQQYYIYPYTFGQGTKVEIKRTVAAPSVFIFPPSDEQLKSGTASVVCLLNNFYPREAKVQWKVDNALQSGNSQESVTEQDSKDSTYSLSSTLTLSKADYEKHKVYACEVTHQGLSSPVTKSFNRGEC

SEQ ID NO: 16 - DNA, 645 bp, Artificial Sequence
  Nucleotide sequence of anti-Her2-domain2-LC
gatatccagatgacccagtctccttccagcctgtctgcctctgtgggcgacagagtgaccatcacatgcaaggcctctcaggacgtgtccatcggcgtggcatggtatcagcagaagcctggcaaggcccctaagctgctgatctactccgcctcctacagatacacaggcgtgccctccagattctccggctctggctctggcacagactttaccctgacaatctccagcctgcagcctgaggacttcgccacctactactgccagcagtactacatctacccctacaccttcggccagggcaccaaggtggaaatcaagagaaccgtggccgctccttccgtgttcatcttcccaccttccgacgagcagctgaagtctggcaccgcttctgtcgtgtgcctgctgaacaacttctaccctcgggaagccaaggtgcagtggaaggtggacaatgccctgcagtccggcaactcccaagagtctgtgaccgagcaggactccaaggacagcacctatagcctgtcctccacactgaccctgtccaaggccgactacgagaagcacaaggtgtacgcctgcgaagtgacccatcagggcctgtctagtcccgtgaccaagtctttcaaccggggcgagtgttga

SEQ ID NO: 17 - protein, 481 aa, Artificial Sequence
  Amino acid sequence of anti-Her2-scFv-VL-VH-Fc
DIQMTQSPSSLSASVGDRVTITCRASQDVNTAVAWYQQKPGKAPKLLIYSASFLYSGVPSRFSGSRSGTDFTLTISSLQPEDFATYYCQQHYTTPPTFGQGTKVEIKGGSGGGSGGGSGGGSGGGSGEVQLVESGGGLVQPGGSLRLSCAASGFNIKDTYIHWVRQAPGKGLEWVARIYPTNGYTRYADSVKGRFTISADTSKNTAYLQMNSLRAEDTAVYYCSRWGGDGFYAMDYWGQGTLVTVSSAAEPKSSDKTHTCPPCPAPELLGGPSVFLFPPKPKDTLMISRTPEVTCVVVDVSHEDPEVKFNWYVDGVEVHNAKTKPREEQYNSTYRVVSVLTVLHQDWLNGKEYKCKVSNKALPAPIEKTISKAKGQPREPQVYTLPPSRDELTKNQVSLICLVKGFYPSDIAVEWESNGQPENRYMTWPPVLDSDGSFFLYSKLTVDKSRWQQGNVFSCSVMHEALHNHYTQKSLSLSPGK

SEQ ID NO: 18 - DNA, 1443 bp, Artificial Sequence
  Nucleotide sequence of anti-Her2-scFv-VL-VH-Fc
gatatccagatgacccagtccccttcctcactgtctgcctccgtgggagacagagtgacaatcacctgcagagcttcccaggatgtgaacaccgcagtggcctggtaccagcagaagcctggcaaggctcctaagctgctgatctactctgcttccttcctgtactccggcgtcccttctcggttctctggctcccggtctggcaccgactttaccctgaccatctccagcctgcagcctgaagacttcgccacctactactgccagcagcactacaccactccacccaccttcggtcagggcaccaaggtcgagatcaagggcggctccggcgggggctccggcggcggctctggcggcggaagcggaggcggaagtggcgaagtgcaactggtcgagtctggaggcggcctggttcagcctggcggaagcctacggctgtcttgcgccgcctctggctttaacatcaaggacacctacatccactgggtgcggcaggctcccggcaagggcctggaatgggtggccagaatctaccctaccaatggctacaccagatacgccgattctgtgaaaggtagattcacaatctccgccgacacctccaagaataccgcctacctgcagatgaactccctgagagccgaggatacagctgtctactactgttccagatggggcggcgatggcttctacgccatggactactggggccagggcacactggtgaccgtgtcctccgctgctgagcctaagtcctccgacaaaacccacacctgtcccccttgtcctgctccagaactcctgggcggcccttccgtgtttctgttccccccgaagcctaaagataccctgatgatctctcgcaccccagaagtgacatgcgtggtagtcgacgtgtctcatgaggaccctgaggtgaagttcaactggtatgtggacggcgtggaagtgcacaacgccaagaccaagcctagagaagagcagtacaactctacctaccgggtggtgtctgtgctgacagtgctgcaccaggactggctgaacggcaaagagtacaagtgcaaggtgtccaacaaggccctgcctgctcccatcgagaagaccatttctaaggccaagggacagcccagagaacctcaagtgtataccctgcctcctagccgggacgagctgaccaagaaccaggtgtccctgatctgcctggtgaagggcttctaccccagcgacatcgccgtggagtgggagtccaacggccaacctgagaaccggtacatgacctggcctcctgtgctggactccgacggcagcttcttcctgtactctaagctgaccgtggacaagagtagatggcagcaaggcaacgtgttctcctgctcggtgatgcacgaggctctgcataaccactacacccagaaatccctgtctttgagccctggcaag

SEQ ID NO: 19 - protein, 448 aa, Artificial Sequence
  Amino acid sequence of anti-Her2-domain2-HC-Fc-2
EVQLVESGGGLVQPGGSLRLSCAASGFTFTDYTMDWVRQAPGKGLEWVADVNPNSGGSIYNQRFKGRFTLSVDRSKNTLYLQMNSLRAEDTAVYYCARNLGPSFYFDYWGQGTLVTVSSASTKGPSVFPLAPSSKSTSGGTAALGCLVKDYFPEPVTVSWNSGALTSGVHTFPAVLQSSGLYSLSSVVTVPSSSLGTQTYICNVNHKPSNTKVDKKVEPKSCDKTHTCPPCPAPELLGGPSVFLFPPKPKDTLMISRTPEVTCVVVDVSHEDPEVKFNWYVDGVEVHNAKTKPREEQYNSTYRVVSVLTVLHQDWLNGKEYKCKVSNKALPAPIEKTISKAKGQPREPQVYVYPPSRDELTKNQVSLTCLVKGFYPSDIAVEWESNGQPENNYKTTPPVLDSDGSFALVSKLTVDKSRWQQGNVFSCSVMHEALHNRFTQKSLSLSPG

SEQ ID NO: 20 - DNA, 1344 bp, Artificial Sequence
  Nucleotide sequence of anti-Her2-domain2-HC-Fc-2
gaggtgcagctggtcgagtctggaggaggtctggtgcagcctggaggctctctgcggctgtcctgtgccgcttctggcttcaccttcaccgactacaccatggactgggtgcggcaggcccctggcaaggggctggaatgggtggccgacgtgaatcctaactctggcggctccatctacaaccagcggttcaagggcagattcacactgtccgtggacagatccaagaacaccctgtacctgcagatgaacagcctgagagccgaggacaccgctgtgtactactgcgcccggaacctgggacccagcttctacttcgactactggggccaaggcaccctggtcaccgtgtccagcgccagcaccaaaggccctagtgtctttcctctggctcccagctctaagtccacctccggcggcaccgctgctctgggctgtctggtgaaggactatttccctgagcctgtgaccgtctcttggaactccggcgctctgacctctggcgtgcatacctttcccgccgtgctgcagtccagcggcctgtactctttgtcttctgtcgtgacagtgccttcttcctctctcggcacacagacctacatctgcaacgtgaaccacaagccatctaacaccaaagtggacaagaaggtggaacccaagagctgcgacaaaacccacacctgtccaccttgtcctgcccctgagctgctgggcggaccttccgtgttcctgttcccccctaagcctaaggatacactgatgatctccagaacccccgaggtgacctgcgtggtggtggatgtttcccatgaagatcctgaagtgaagttcaactggtacgtggacggcgtggaagtgcacaacgccaagaccaagcctagagaggaacagtacaactctacctacagagtggtttctgtgctcactgtgctgcaccaggattggctgaacggcaaagagtacaagtgcaaggtgtccaacaaggccctgcctgctcctatcgagaagaccatcagcaaggctaagggccagcctcgcgaacctcaggtgtacgtgtatcctccttcccgggacgagctgaccaagaaccaagtgtctctgacctgcctggtgaaaggcttctacccctccgacatcgccgtggaatgggagtccaatggccagcccgagaacaactacaagaccacccctccagtgctggactccgatggctccttcgccctggtgtccaagctgacagtagacaagtctagatggcagcagggcaacgtgttctcctgctccgtgatgcacgaggccctgcacaatagattcacacagaagtccctgtctctgtcccctggc

SEQ ID NO: 21 - protein, 480 aa, Artificial Sequence
  Amino acid sequence of b-anti-Her2-scFv-VH-K30E-Fc
EVQLVESGGGLVQPGGSLRLSCAASGFNIEDTYIHWVRQAPGKGLEWVARIYPTNGYTRYADSVKGRFTISADTSKNTAYLQMNSLRAEDTAVYYCSRWGGDGFYAMDYWGQGTLVTVSSGGGGSGGGGSGGGGSGGGGSDIQMTQSPSSLSASVGDRVTITCRASQDVNTAVAWYQQKPGKAPKLLIYSASFLYSGVPSRFSGSRSGTDFTLTISSLQPEDFATYYCQQHYTTPPTFGQGTKVEIKGEPKSSDKTHTCPPCPAPELLGGPSVFLFPPKPKDTLMISRTPEVTCVVVDVSHEDPEVKFNWYVDGVEVHNAKTKPREEQYNSTYRVVSVLTVLHQDWLNGKEYKCKVSNKALPAPIEKTISKAKGQPREPQVYTLPPCREEMTKNQVSLWCLVKGFYPSDIAVEWESNGQPENNYKTTPPVLDSDGSFFLYSKLTVDKSRWQQGNVFSCSVMHEALHNHYTQKSLSLSPGK

SEQ ID NO: 22 - DNA, 1443 bp, Artificial Sequence
  Nucleotide sequence of b-anti-Her2-scFv-VH-K30E-Fc
gaggtgcaactggtggaatccggcgggggactggtccaacctggagggagcctgcggctgtcttgcgccgcctctggcttcaacatcgaggatacctacatccactgggtgcggcaggcccctggcaagggcctggaatgggtcgctagaatctaccctaccaacggctacaccagatacgccgactctgtaaagggcagattcaccatctctgccgatacatctaagaacaccgcctacctgcagatgaactccctgagagccgaggacaccgccgtgtactactgctcccggtggggcggtgacggcttttacgccatggactactggggacaaggcacacttgttacggtgtcctctggaggcggcggctccggcggcggcggctctggcggaggcggctctggcggcggcggatctgatatccagatgacccagtctcctagctccctctccgcctccgtgggcgacagagtgacaatcacctgcagagcttctcaggacgtgaacaccgctgtggcctggtaccagcagaagcctggcaaggcccctaagctgctgatctactctgcttccttcctgtactccggcgtgcccagccggttctccggctctcggtccggcaccgacttcactctgaccatctccagcctgcagcctgaagatttcgccacctactactgccagcagcactacaccacccctcccaccttcggccagggcaccaaagtggagatcaagggcgagcccaagtcctccgataaaacccacacctgtcctccttgccctgcccctgaactactgggcggcccttctgtgttcctgttccctcctaagcccaaggacaccctgatgatctctagaacccctgaagtgacctgcgtggtggtggatgtgtctcacgaggaccctgaggtcaagttcaactggtacgtggacggcgtggaagtgcataacgccaagaccaagcctagagaagagcagtacaactccacctacagagtggtctccgtgctgaccgtgctgcaccaggactggctgaacggcaaagagtacaagtgcaaggtgtccaacaaggctctgcctgctcctatcgagaagacaatctccaaggccaaaggccagcctcgggagcctcaggtgtacaccctgcctccttgtagagaggaaatgaccaagaaccaggtgtctctgtggtgcctggtgaagggcttctacccatccgacatcgccgtcgagtgggagtccaacggacagcccgagaacaactacaagactaccccacctgtgctggactccgatggctccttcttcctgtactccaagctgaccgtggacaagtccagatggcagcagggcaacgtgttctcctgctccgtgatgcacgaggccctgcacaaccactacacccagaaatccctgtctctgtcccctggcaagtga

SEQ ID NO: 23 - protein, 480 aa, Artificial Sequence
  Amino acid sequence of b-anti-Her2-scFv-VL-F53Y-Fc
EVQLVESGGGLVQPGGSLRLSCAASGFNIKDTYIHWVRQAPGKGLEWVARIYPTNGYTRYADSVKGRFTISADTSKNTAYLQMNSLRAEDTAVYYCSRWGGDGFYAMDYWGQGTLVTVSSGGGGSGGGGSGGGGSGGGGSDIQMTQSPSSLSASVGDRVTITCRASQDVNTAVAWYQQKPGKAPKLLIYSASYLYSGVPSRFSGSRSGTDFTLTISSLQPEDFATYYCQQHYTTPPTFGQGTKVEIKGEPKSSDKTHTCPPCPAPELLGGPSVFLFPPKPKDTLMISRTPEVTCVVVDVSHEDPEVKFNWYVDGVEVHNAKTKPREEQYNSTYRVVSVLTVLHQDWLNGKEYKCKVSNKALPAPIEKTISKAKGQPREPQVYTLPPCREEMTKNQVSLWCLVKGFYPSDIAVEWESNGQPENNYKTTPPVLDSDGSFFLYSKLTVDKSRWQQGNVFSCSVMHEALHNHYTQKSLSLSPGK

SEQ ID NO: 24 - DNA, 1443 bp, Artificial Sequence
  Nucleotide sequence of b-anti-Her2-scFv-VL-F53Y-Fc
gaggtgcaactggtggaatccggcgggggactggtccaacctggagggagcctgcggctgtcttgcgccgcctctggcttcaacatcaaggatacctacatccactgggtgcggcaggcccctggcaagggcctggaatgggtcgctagaatctaccctaccaacggctacaccagatacgccgactctgtaaagggcagattcaccatctctgccgatacatctaagaacaccgcctacctgcagatgaactccctgagagccgaggacaccgccgtgtactactgctcccggtggggcggtgacggcttttacgccatggactactggggacaaggcacacttgttacggtgtcctctggaggcggcggctccggcggcggcggctctggcggaggcggctctggcggcggcggatctgatatccagatgacccagtctcctagctccctctccgcctccgtgggcgacagagtgacaatcacctgcagagcttctcaggacgtgaacaccgctgtggcctggtaccagcagaagcctggcaaggcccctaagctgctgatctactctgcttcctacctgtactccggcgtgcccagccggttctccggctctcggtccggcaccgacttcactctgaccatctccagcctgcagcctgaagatttcgccacctactactgccagcagcactacaccacccctcccaccttcggccagggcaccaaagtggagatcaagggcgagcccaagtcctccgataaaacccacacctgtcctccttgccctgcccctgaactactgggcggcccttctgtgttcctgttccctcctaagcccaaggacaccctgatgatctctagaacccctgaagtgacctgcgtggtggtggatgtgtctcacgaggaccctgaggtcaagttcaactggtacgtggacggcgtggaagtgcataacgccaagaccaagcctagagaagagcagtacaactccacctacagagtggtctccgtgctgaccgtgctgcaccaggactggctgaacggcaaagagtacaagtgcaaggtgtccaacaaggctctgcctgctcctatcgagaagacaatctccaaggccaaaggccagcctcgggagcctcaggtgtacaccctgcctccttgtagagaggaaatgaccaagaaccaggtgtctctgtggtgcctggtgaagggcttctacccatccgacatcgccgtcgagtgggagtccaacggacagcccgagaacaactacaagactaccccacctgtgctggactccgatggctccttcttcctgtactccaagctgaccgtggacaagtccagatggcagcagggcaacgtgttctcctgctccgtgatgcacgaggccctgcacaaccactacacccagaaatccctgtctctgtcccctggcaagtga

SEQ ID NO: 25 - protein, 480 aa, Artificial Sequence
  Amino acid sequence of anti-Her2-scFv-VH-VL-Fc
EVQLVESGGGLVQPGGSLRLSCAASGFNIKDTYIHWVRQAPGKGLEWVARIYPTNGYTRYADSVKGRFTISADTSKNTAYLQMNSLRAEDTAVYYCSRWGGDGFYAMDYWGQGTLVTVSSGGGGSGGGGSGGGGSGGGGSDIQMTQSPSSLSASVGDRVTITCRASQDVNTAVAWYQQKPGKAPKLLIYSASFLYSGVPSRFSGSRSGTDFTLTISSLQPEDFATYYCQQHYTTPPTFGQGTKVEIKGEPKSSDKTHTCPPCPAPELLGGPSVFLFPPKPKDTLMISRTPEVTCVVVDVSHEDPEVKFNWYVDGVEVHNAKTKPREEQYNSTYRVVSVLTVLHQDWLNGKEYKCKVSNKALPAPIEKTISKAKGQPREPQVYTLPPCREEMTKNQVSLWCLVKGFYPSDIAVEWESNGQPENNYKTTPPVLDSDGSFFLYSKLTVDKSRWQQGNVFSCSVMHEALHNHYTQKSLSLSPGK

SEQ ID NO: 26 - DNA, 1440 bp, Artificial Sequence
  Nucleotide sequence of anti-Her2-scFv-VH-VL-Fc
gaggtgcaactggtggaatccggcgggggactggtccaacctggagggagcctgcggctgtcttgcgccgcctctggcttcaacatcaaggatacctacatccactgggtgcggcaggcccctggcaagggcctggaatgggtcgctagaatctaccctaccaacggctacaccagatacgccgactctgtaaagggcagattcaccatctctgccgatacatctaagaacaccgcctacctgcagatgaactccctgagagccgaggacaccgccgtgtactactgctcccggtggggcggtgacggcttttacgccatggactactggggacaaggcacacttgttacggtgtcctctggaggcggcggctccggcggcggcggctctggcggaggcggctctggcggcggcggatctgatatccagatgacccagtctcctagctccctctccgcctccgtgggcgacagagtgacaatcacctgcagagcttctcaggacgtgaacaccgctgtggcctggtaccagcagaagcctggcaaggcccctaagctgctgatctactctgcttccttcctgtactccggcgtgcccagccggttctccggctctcggtccggcaccgacttcactctgaccatctccagcctgcagcctgaagatttcgccacctactactgccagcagcactacaccacccctcccaccttcggccagggcaccaaagtggagatcaagggcgagcccaagtcctccgataaaacccacacctgtcctccttgccctgcccctgaactactgggcggcccttctgtgttcctgttccctcctaagcccaaggacaccctgatgatctctagaacccctgaagtgacctgcgtggtggtggatgtgtctcacgaggaccctgaggtcaagttcaactggtacgtggacggcgtggaagtgcataacgccaagaccaagcctagagaagagcagtacaactccacctacagagtggtctccgtgctgaccgtgctgcaccaggactggctgaacggcaaagagtacaagtgcaaggtgtccaacaaggctctgcctgctcctatcgagaagacaatctccaaggccaaaggccagcctcgggagcctcaggtgtacaccctgcctccttgtagagaggaaatgaccaagaaccaggtgtctctgtggtgcctggtgaagggcttctacccatccgacatcgccgtcgagtgggagtccaacggacagcccgagaacaactacaagactaccccacctgtgctggactccgatggctccttcttcctgtactccaagctgaccgtggacaagtccagatggcagcagggcaacgtgttctcctgctccgtgatgcacgaggccctgcacaaccactacacccagaaatccctgtctctgtcccctggcaag

SEQ ID NO: 27 - protein, 10 aa, Artificial Sequence
  UNSURE (5): Xaa is K or E
GFNIXDTYIH

SEQ ID NO: 28 - protein, 17 aa, Mus musculus
RIYPTNGYTRYADSVKG

SEQ ID NO: 29 - protein, 12 aa, Mus musculus
WGGDGFYAMDYW

SEQ ID NO: 30 - protein, 13 aa, Mus musculus
CRASQDVNTAVAW

SEQ ID NO: 31 - protein, 7 aa, Artificial Sequence
SASYLYS

SEQ ID NO: 32 - protein, 9 aa, Mus musculus
QQHYTTPPT

SEQ ID NO: 33 - protein, 7 aa, Mus musculus
SASFLYS

SEQ ID NO: 34 - protein, 7 aa, Artificial Sequence
  UNSURE (4): Xaa is F or Y
SASXLYS

SEQ ID NO: 35 - protein, 120 aa, Artificial Sequence
EVQLVESGGGLVQPGGSLRLSCAASGFNIEDTYIHWVRQAPGKGLEWVARIYPTNGYTRYADSVKGRFTISADTSKNTAYLQMNSLRAEDTAVYYCSRWGGDGFYAMDYWGQGTLVTVSS

SEQ ID NO: 36 - protein, 107 aa, Artificial Sequence
DIQMTQSPSSLSASVGDRVTITCRASQDVNTAVAWYQQKPGKAPKLLIYSASYLYSGVPSRFSGSRSGTDFTLTISSLQPEDFATYYCQQHYTTPPTFGQGTKVEIK

SEQ ID NO: 37 - protein, 119 aa, Artificial Sequence [sequence omitted]

SEQ ID NO: 38 - protein, 107 aa, Artificial Sequence [sequence omitted]

SEQ ID NO: 39 - protein, 107 aa, Artificial Sequence [sequence omitted]

SEQ ID NO: 40 - protein, 120 aa, Artificial Sequence [sequence omitted]

SEQ ID NO: 41 - protein, 120 aa, Artificial Sequence
  UNSURE (30): Xaa is K or E
EVQLVESGGGLVQPGGSLRLSCAASGFNIXDTYIHWVRQAPGKGLEWVARIYPTNGYTRYADSVKGRFTISADTSKNTAYLQMNSLRAEDTAVYYCSRWGGDGFYAMDYWGQGTLVTVSS

SEQ ID NO: 42 - protein, 107 aa, Artificial Sequence
  UNSURE (53): Xaa is F or Y
DIQMTQSPSSLSASVGDRVTITCRASQDVNTAVAWYQQKPGKAPKLLIYSASXLYSGVPSRFSGSRSGTDFTLTISSLQPEDFATYYCQQHYTTPPTFGQGTKVEIK

SEQ ID NO: 43 - protein, 10 aa, Artificial Sequence
GFNIEDTYIH

SEQ ID NO: 44 - protein, 10 aa, Mus musculus
GFNIKDTYIH

SEQ ID NO: 45 - protein, 10 aa, Mus musculus
GFTFTDYTMD

SEQ ID NO: 46 - protein, 17 aa, Mus musculus
DVNPNSGGSIYNQRFKG

SEQ ID NO: 47 - protein, 10 aa, Mus musculus
NLGPSFYFDY

SEQ ID NO: 48 - protein, 11 aa, Mus musculus
KASQDVSIGVA

SEQ ID NO: 49 - protein, 7 aa, Mus musculus
SASYRYT

SEQ ID NO: 50 - protein, 9 aa, Mus musculus
QQYYIYPYT